European Patent Specification EP 3 568 204 B1, published August 30, 2023. Title: Pharmaceutical Combinations. Applicant: Novartis AG Hao, Huaixiang LaMarche , Matthew  J Li, Fang Wang, Hui-Qin Alghalandis, Leila Dardaei Engelman, Jeffrey A. The sequence listing filed with the application follows.

SEQUENCE LISTING (1 sequence)

SEQ ID NO: 1 - protein, 20 aa, Artificial Sequence
  biphosphorylated peptide derived from insulin receptor substrate-1 (IRS-1)
  MOD_RES (3)..(3): PHOSPHORYLATED TYROSINE
  MOD_RES (9)..(10): Pegylated (dPEG8) between valine residue 9 and leucine residue 10
  MOD_RES (13)..(13): PHOSPHORYLATED TYROSINE
  MOD_RES (20)..(20): AMIDATED Lysine
LNYIDLDLVLSTYASINFQK